European Patent Specification EP 3 889 182 B1, published May 22, 2024. Title: ANTIGEN BINDING CONSTRUCTS TO CD8. Applicant: Imaginab, Inc. The sequence listing filed with the application follows.

SEQUENCE LISTING (81 sequences)

SEQ ID NO: 1 - protein, 118 aa, Murine
EVQLQQSGAELVKPGASVKLSCTASGFNIKDTYIHFVRQRPEQGLEWIGRIDPANDNTLYASKFQGKATITADTSSNTAYMHLCSLTSGDTAVYYCGRGYGYYVFDHWGQGTTLTVSS

SEQ ID NO: 2 - protein, 120 aa, Homo sapiens [sequence omitted]

SEQ ID NO: 3 - protein, 118 aa, Artificial Sequence
  Antigen binding construct or fragment thereof
EVQLVESGGGLVQPGGSLRLSCAASGFNIKDTYIHWVRQAPGKGLEWVARIDPANDNTLYASKFQGRATISADTSKNTAYLQMNSLRAEDTAVYYCGRGYGYYVFDHWGQGTLVTVSS

SEQ ID NO: 4 - protein, 118 aa, Murine
QVQLQQSGAELVKPGASVKLSCTASGFNIKDTYIHFVRQRPEQGLEWIGRIDPANDNTLYASKFQGKATITADTSSNTAYMHLCSLTSGDTAVYYCGRGYGYYVFDHWGQGTTLTVSS

SEQ ID NO: 5 - protein, 115 aa, Homo sapiens
EVQLVQSGAEVKKPGATVKISCKVSGYTFTDYYMHWVQQAPGKGLEWMGLVDPEDGETIYAEKFQGRVTITADTSTDTAYMELSSLRSEDTAVYYCATAEYFQHWGQGTLVTVSS

SEQ ID NO: 6 - protein, 118 aa, Artificial Sequence
  Antigen binding construct or fragment thereof
QVQLVQSGAEVKKPGATVKISCKVSGFNIKDTYIHWVQQAPGKGLEWMGRIDPANDNTLYASKFQGRVTITADTSTDTAYMELSSLRSEDTAVYYCARGYGYYVFDHWGQGTLVTVSS

SEQ ID NO: 7 - protein, 107 aa, Murine
DVQINQSPSFLAASPGETITINCRTSRSISQYLAWYQEKPGKTNKLLIYSGSTLQSGIPSRFSGSGSGTDFTLTISGLEPEDFAMYYCQQHNENPLTFGAGTKLELK

SEQ ID NO: 8 - protein, 107 aa, Homo sapiens
DIQMTQSPSSLSASVGDRVTITCRASQGISNYLAWYQQKPGKVPKLLIYAASTLQSGVPSRFSGSGSGTDFTLTISSLQPEDVATYYCQKYNSAPLTFGGGTKVEIK

SEQ ID NO: 9 - protein, 107 aa, Artificial Sequence
  Antigen binding construct or fragment thereof
DVQITQSPSSLSASVGDRVTITCRTSRSISQYLAWYQQKPGKVPKLLIYSGSTLQSGVPSRFSGSGSGTDFTLTISSLQPEDVATYYCQQHNENPLTFGGGTKVEIK

SEQ ID NO: 10 - DNA, 768 bp, Artificial Sequence
  Antigen binding construct or fragment thereof
atggagaccgatacactgctgctgtgggtgctgctgctctgggtccctggcagcacaggagacatccagatgacacagagccctagctccctgagcgcttccgtgggagatagggtgaccatcacatgccggacctccaggtccatctcccagtacctggcctggtaccagcagaagcccggcaaggtgcccaagctgctcatctatagcggcagcaccctgcagagcggagtgccttcccggttttccggatccggctccggcacagactttaccctgaccatctccagcctgcagcctgaggatgtcgccacctactactgccaacagcacaacgagaaccccctgaccttcggcggcggaaccaaggtcgagatcaagggaggaggctccggaggaggaggccaagtgcagctggtccaatccggcgccgaagtgaaaaagcccggcgccaccgtgaagatcagctgcaaggtgtccggcttcaacatcaaggacacctatatccactgggtccagcaagcccccggaaaaggcctggagtggatgggacggattgaccccgccaacgacaacacactctatgcctccaagttccagggcagggtgacaatcaccgccgacaccagcaccgacacagcttatatggagctgtcctccctccggtccgaggataccgccgtctactactgcgccaggggctacggctactacgtgtttgaccactggggccagggcaccctggtgacagtgtccagcggaggctgc

SEQ ID NO: 11 - DNA, 768 bp, Artificial Sequence
  Antigen binding construct or fragment thereof
atggagaccgacaccctgctgctctgggtcctcctgctgtgggtgcctggcagcacaggacaggtgcaactggtgcagagcggcgccgaggtcaagaaacctggcgccaccgtgaagatcagctgcaaggtgtccggcttcaacatcaaggacacctacatccactgggtccaacaagcccccggaaagggcctggaatggatgggccggattgaccccgccaacgacaacaccctctatgccagcaagttccagggcagggtcaccatcaccgccgacaccagcaccgacaccgcctacatggagctgagcagcctgcggagcgaagacaccgccgtgtactactgcgccaggggctacggctactacgtcttcgaccattggggacagggcaccctcgtgacagtgtccagcggaggaggatccggcggaggaggagatatccagatgacccagagcccttccagcctgtccgcttccgtgggagatcgggtgaccatcacatgcaggacctccaggtccatctcccagtacctggcctggtaccaacagaagcccggcaaggtgcccaagctgctgatctacagcggcagcacactgcaatccggcgtcccttcccggttttccggatccggatccggcaccgacttcaccctgaccatcagctccctgcaacccgaggacgtggccacctactactgtcagcagcacaacgagaaccccctcacctttggcggcggaaccaaggtcgagatcaagggcggctgc

SEQ ID NO: 12 - protein, 253 aa, Artificial Sequence
  Antigen binding construct or fragment thereof
METDTLLLWVLLLWVPGSTGDIQMTQSPSSLSASVGDRVTITCRTSRSISQYLAWYQQKPGKVPKLLIYSGSTLQSGVPSRFSGSGSGTDFTLTISSLQPEDVATYYCQQHNENPLTFGGGTKVEIKSGGGGQVQLVQSGAEVKKPGATVKISCKVSGFNIKDTYIHWVQQAPGKGLEWMGRIDPANDNTLYASKFQGRVTITADTSTDTAYMELSSLRSEDTAVYYCARGYGYYVFDHWGQGTLVTVSSGGC

SEQ ID NO: 13 - protein, 253 aa, Artificial Sequence
  Antigen binding construct or fragment thereof
METDTLLLWVLLLWVPGSTGQVQLVQSGAEVKKPGATVKISCKVSGFNIKDTYIHWVQQAPGKGLEWMGRIDPANDNTLYASKFQGRVTITADTSTDTAYMELSSLRSEDTAVYYCARGYGYYVFDHWGQGTLVTVSSSGGGGDIQMTQSPSSLSASVGDRVTITCRTSRSISQYLAWYQQKPGKVPKLLIYSGSTLQSGVPSRFSGSGSGTDFTLTISSLQPEDVATYYCQQHNENPLTFGGGTKVEIKGGC

SEQ ID NO: 14 - protein, 256 aa, Artificial Sequence
  Antigen binding construct or fragment thereof
METDTLLLWVLLLWVPGSTGDIQMTQSPSSLSASVGDRVTITCRTSRSISQYLAWYQQKPGKVPKLLIYSGSTLQSGVPSRFSGSGSGTDFTLTISSLQPEDVATYYCQQHNENPLTFGGGTKVEIKGGGSGGGGQVQLVQSGAEVKKPGATVKISCKVSGFNIKDTYIHWVQQAPGKGLEWMGRIDPANDNTLYASKFQGRVTITADTSTDTAYMELSSLRSEDTAVYYCARGYGYYVFDHWGQGTLVTVSSGGC

SEQ ID NO: 15 - protein, 256 aa, Artificial Sequence
  Antigen binding construct or fragment thereof
METDTLLLWVLLLWVPGSTGQVQLVQSGAEVKKPGATVKISCKVSGFNIKDTYIHWVQQAPGKGLEWMGRIDPANDNTLYASKFQGRVTITADTSTDTAYMELSSLRSEDTAVYYCARGYGYYVFDHWGQGTLVTVSSGGGSGGGGDIQMTQSPSSLSASVGDRVTITCRTSRSISQYLAWYQQKPGKVPKLLIYSGSTLQSGVPSRFSGSGSGTDFTLTISSLQPEDVATYYCQQHNENPLTFGGGTKVEIKGGC

SEQ ID NO: 16 - protein, 394 aa, Artificial Sequence
  Antigen binding construct or fragment thereof
METDTLLLWVLLLWVPGSTGDVQINQSPSFLAASPGETITINCRTSRSISQYLAWYQEKPGKTNKLLIYSGSTLQSGIPSRFSGSGSGTDFTLTISGLEPEDFAMYYCQQHNENPLTFGAGTKLELKGSTSGGGSGGGSGGGGSSEVQLQQSGAELVKPGASVKLSCTASGFNIKDTYIHFVRQRPEQGLEWIGRIDPANDNTLYASKFQGKATITADTSSNTAYMHLSSLTSGDTAVYYCGRGYGYYVFDHWGQGTTLTVSSEPKSCDKTHTCPPCGGGSSGGGSGGQPREPQVYTLPPSRDELTKNQVSLTCLVKGFYPSDIAVEWESNGQPENNYKTTPPVLDSDGSFFLYSKLTVDKSRWQQGNVFSCSVMHEALHNHYTQKSLSLSPGK

SEQ ID NO: 17 - DNA, 1185 bp, Artificial Sequence
  Antigen binding construct or fragment thereof
atggagacagacaccctgctcctgtgggtgctgctcctctgggtccctggatccaccggcgatgtccagatcaaccaaagccccagctttctggctgcctcccctggagagacaatcaccatcaattgccggaccagccggagcatttcccagtacctcgcctggtaccaggaaaagcctggcaagaccaacaagctgctgatctactccggctccacactccagagcggcattccctccaggtttagcggatccggatccggaaccgacttcacactcaccatctccggcctggagcccgaggacttcgccatgtattattgccagcagcacaatgagaaccccctgaccttcggcgctggcaccaagctggagctgaaaggctccaccagcggaggcggatccggaggaggaagcggcggcggaggctcctccgaagtgcagctgcaacagagcggcgccgaactggtgaagcctggagcttccgtgaaactcagctgtaccgccagcggcttcaacatcaaggatacctacatccacttcgtgcggcaaaggcctgagcagggcctggaatggatcggcaggatcgaccccgccaacgacaacaccctctacgcctccaagttccaaggcaaggccacaatcaccgctgatacaagctccaacaccgcctacatgcacctcagctccctgaccagcggagacaccgccgtgtactactgcggacggggatacggctactatgtgttcgaccactggggccaaggcaccacactcaccgtgtcctccgagcccaagtcctgcgacaagacacacacctgtcccccttgtggaggaggatcctccggaggcggctccggcggacagcctagggagccccaggtgtacacactgcccccttccagggacgaactcaccaagaaccaggtgtccctgacctgcctggtgaagggattctaccccagcgacatcgccgtggagtgggagtccaacggccaacccgagaacaattacaagaccaccccccctgtgctcgattccgacggctccttcttcctgtactccaagctcaccgtggacaagtcccggtggcaacagggcaatgtgttctcctgcagcgtcatgcacgaggccctgcataaccactacacccagaaatccctcagcctctcccctggaaaatga

SEQ ID NO: 18 - protein, 394 aa, Artificial Sequence
  Antigen binding construct or fragment thereof
METDTLLLWVLLLWVPGSTGEVQLQQSGAELVKPGASVKLSCTASGFNIKDTYIHFVRQRPEQGLEWIGRIDPANDNTLYASKFQGKATITADTSSNTAYMHLSSLTSGDTAVYYCGRGYGYYVFDHWGQGTTLTVSSGSTSGGGSGGGSGGGGSSDVQINQSPSFLAASPGETITINCRTSRSISQYLAWYQEKPGKTNKLLIYSGSTLQSGIPSRFSGSGSGTDFTLTISGLEPEDFAMYYCQQHNENPLTFGAGTKLELKEPKSCDKTHTCPPCGGGSSGGGSGGQPREPQVYTLPPSRDELTKNQVSLTCLVKGFYPSDIAVEWESNGQPENNYKTTPPVLDSDGSFFLYSKLTVDKSRWQQGNVFSCSVMHEALHNHYTQKSLSLSPGK

SEQ ID NO: 19 - DNA, 1185 bp, Artificial Sequence
  Antigen binding construct or fragment thereof
atggagaccgacacactcctgctctgggtgctcctgctgtgggtgcctggcagcacaggagaagtgcagctgcagcagtccggcgccgaactcgtcaaacccggagcctccgtcaaactgtcctgcacagccagcggcttcaacatcaaggacacctacatccatttcgtgcggcaaaggcctgaacagggactcgagtggatcggcaggatcgaccccgccaacgacaataccctctacgcctccaagttccagggaaaggccaccattaccgccgacacatccagcaacaccgcctacatgcacctcagctccctgacatccggcgacaccgccgtgtactactgcggcaggggctacggctactacgtgtttgaccactggggccagggaacaaccctgaccgtgtccagcggctccacctccggaggcggaagcggcggaggatccggaggaggaggctcctccgacgtgcaaatcaaccagtcccctagcttcctggccgctagccctggcgagacaatcacaatcaattgtcggaccagccggtccatctcccagtatctggcctggtaccaggagaagcccggcaagacaaacaagctgctcatctacagcggcagcaccctccaatccggcatcccttcccggtttagcggctccggatccggaaccgactttaccctgaccatcagcggcctggaacccgaggatttcgccatgtactactgccagcagcacaacgagaatcccctgacctttggagccggcacaaagctcgagctgaaggagcccaagagctgcgacaaaacccacacctgtcccccttgcggaggaggatcctccggcggcggaagcggaggacaacccagggagccccaggtctacaccctgcctcctagccgggacgaactgacaaagaaccaggtgtccctgacctgtctcgtcaagggcttctacccttccgacatcgccgtcgagtgggaaagcaacggccagcccgagaacaattacaagaccacaccccccgtcctggacagcgatggcagcttcttcctctactccaagctgaccgtggacaagagccggtggcaacaaggcaacgtgttctcctgcagcgtcatgcatgaggccctgcacaatcactacacccagaagagcctgagcctctcccccggcaagtga

SEQ ID NO: 20 - protein, 394 aa, Artificial Sequence
  Antigen binding construct or fragment thereof
METDTLLLWVLLLWVPGSTGDIQMTQSPSSLSASVGDRVTITCRTSRSISQYLAWYQQKPGKVPKLLIYSGSTLQSGVPSRFSGSGSGTDFTLTISSLQPEDVATYYCQQHNENPLTFGGGTKVEIKGSTSGGGSGGGSGGGGSSQVQLVQSGAEVKKPGATVKISCKVSGFNIKDTYIHWVQQAPGKGLEWMGRIDPANDNTLYASKFQGRVTITADTSTDTAYMELSSLRSEDTAVYYCARGYGYYVFDHWGQGTLVTVSSEPKSCDKTHTCPPCGGGSSGGGSGGQPREPQVYTLPPSRDELTKNQVSLTCLVKGFYPSDIAVEWESNGQPENNYKTTPPVLDSDGSFFLYSKLTVDKSRWQQGNVFSCSVMHEALHNHYTQKSLSLSPGK

SEQ ID NO: 21 - DNA, 1185 bp, Artificial Sequence
  Antigen binding construct or fragment thereof
atggagacagacaccctcctgctgtgggtcctgctgctgtgggtgcctggcagcacaggagacatccaaatgacccagtcccctagcagcctcagcgcttccgtcggagacagggtcaccatcacatgcaggacctccaggtccatcagccagtatctggcctggtatcagcagaaacccggcaaggtgcctaagctgctgatctacagcggcagcacactccagagcggagtgcccagccggttttccggaagcggatccggaaccgacttcaccctgaccatttccagcctgcaacctgaagacgtggccacctactactgtcagcagcacaacgagaaccccctcaccttcggcggaggcaccaaagtcgagatcaagggcagcaccagcggaggaggaagcggcggaggctccggaggaggaggctcctcccaagtgcagctcgtccaaagcggcgctgaggtgaaaaagcccggcgccacagtcaaaatctcctgcaaggtcagcggcttcaacatcaaggatacctacatccactgggtgcaacaggcccccggcaaaggactcgaatggatgggccggatcgaccctgctaacgacaacacactctacgcctccaagttccagggcagggtgaccatcaccgccgatacctccaccgacacagcctacatggagctgagcagcctgaggtccgaggacaccgccgtctattactgcgcccggggatacggctactacgtgtttgaccattggggacagggaacactcgtgaccgtgagctccgagcccaagagctgcgacaagacccacacatgtcctccttgcggaggaggcagctccggaggcggatccggcggacaacctagggagccccaggtctataccctgccccccagcagggacgagctgacaaagaaccaggtctccctgacctgcctggtgaaaggattctaccccagcgacatcgctgtcgaatgggagtccaacggccagcccgagaacaactacaagacaaccccccccgtgctggattccgacggcagcttcttcctctactccaagctgaccgtcgacaagtccaggtggcagcagggcaacgtgttttcctgctccgtgatgcatgaggccctgcacaaccactacacccagaagtccctgagcctcagccctggcaagtga

SEQ ID NO: 22 - protein, 394 aa, Artificial Sequence
  Antigen binding construct or fragment thereof
METDTLLLWVLLLWVPGSTGQVQLVQSGAEVKKPGATVKISCKVSGFNIKDTYIHWVQQAPGKGLEWMGRIDPANDNTLYASKFQGRVTITADTSTDTAYMELSSLRSEDTAVYYCARGYGYYVFDHWGQGTLVTVSSGSTSGGGSGGGSGGGGSSDIQMTQSPSSLSASVGDRVTITCRTSRSISQYLAWYQQKPGKVPKLLIYSGSTLQSGVPSRFSGSGSGTDFTLTISSLQPEDVATYYCQQHNENPLTFGGGTKVEIKEPKSCDKTHTCPPCGGGSSGGGSGGQPREPQVYTLPPSRDELTKNQVSLTCLVKGFYPSDIAVEWESNGQPENNYKTTPPVLDSDGSFFLYSKLTVDKSRWQQGNVFSCSVMHEALHNHYTQKSLSLSPGK

SEQ ID NO: 23 - DNA, 1185 bp, Artificial Sequence
  Antigen binding construct or fragment thereof
atggagaccgatacactgctgctctgggtgctgctgctgtgggtgcctggaagcaccggacaggtgcaactggtccagtccggcgccgaggtgaaaaagcctggcgccaccgtcaagatctcctgtaaggtgagcggcttcaacatcaaggacacctacatccactgggtgcagcaggctcccggaaagggactggagtggatgggcaggatcgaccctgccaatgacaacaccctctacgccagcaagttccaaggacgggtgaccatcacagccgacacatccaccgacacagcctatatggagctctccagcctgaggtccgaggacaccgccgtgtactactgtgccaggggatacggctattacgtgttcgaccactggggacagggcaccctggtgaccgtgagcagcggaagcaccagcggcggaggcagcggaggcggaagcggcggcggcggatcctccgacattcagatgacccaatccccctccagcctgtccgctagcgtgggagacagggtgacaatcacatgtcggacctccaggtccatcagccaatatctcgcctggtatcagcagaagcccggcaaggtgcccaagctcctgatctacagcggctccaccctccaaagcggagtgccttcccggtttagcggaagcggcagcggcacagactttaccctgacaatcagctccctgcaacctgaggacgtcgccacatactactgccagcagcacaacgagaaccctctcacctttggcggcggcaccaaagtggagatcaaggagcccaaatcctgcgacaagacacacacctgccccccttgtggaggaggcagctccggcggcggcagcggcggacaaccccgggaacctcaggtgtatacactccccccttccagggatgagctgaccaagaaccaagtctccctgacctgtctggtgaaaggcttctacccctccgacatcgctgtcgagtgggagagcaacggccagcccgaaaacaactataagaccaccccccccgtgctcgattccgatggcagcttcttcctgtactccaagctcacagtcgacaagagccggtggcaacagggcaacgtcttctcctgtagcgtcatgcacgaggccctccacaaccactacacccagaagtccctctccctgagccccggaaaatga

SEQ ID NO: 24 - protein, 235 aa, Homo sapiens
MALPVTALLLPLALLLHAARPSQFRVSPLDRTWNLGETVELKCQVLLSNPTSGCSWLFQPRGAAASPTFLLYLSQNKPKAAEGLDTQRFSGKRLGDTFVLTLSDFRRENEGYYFCSALSNSIMYFSHFVPVFLPAKPTTTPAPRPPTPAPTIASQPLSLRPEACRPAAGGAVHTRGLDFACDIYIWAPLAGTCGVLLLSLVITLYCNHRNRRRVCKCPRPVVKSGDKPSLSARYV

SEQ ID NO: 25 - DNA, 60 bp, Artificial Sequence
  Antigen binding construct or fragment thereof
atggaaaccgacaccctgctgctgtgggtgctgctgctctgggtcccaggctccaccggt

SEQ ID NO: 26 - protein, 20 aa, Artificial Sequence
  Antigen binding construct or fragment thereof
METDTLLLWVLLLWVPGSTG

SEQ ID NO: 27 - DNA, 15 bp, Artificial Sequence
  Antigen binding construct or fragment thereof
agtggtggaggaggc

SEQ ID NO: 28 - protein, 5 aa, Artificial Sequence
  Antigen binding construct or fragment thereof
SGGGG

SEQ ID NO: 29 - DNA, 24 bp, Artificial Sequence
  Antigen binding construct or fragment thereof
ggcggagggagtggcggaggcggc

SEQ ID NO: 30 - protein, 8 aa, Artificial Sequence
  Antigen binding construct or fragment thereof
GGGSGGGG

SEQ ID NO: 31 - DNA, 9 bp, Artificial Sequence
  Antigen binding construct or fragment thereof
ggcggctgc

SEQ ID NO: 32 - protein, 3 aa, Artificial Sequence
  Antigen binding construct or fragment thereof
GGC

SEQ ID NO: 33 - DNA, 60 bp, Artificial Sequence; identical to SEQ ID NO: 25
  Antigen binding construct or fragment thereof

SEQ ID NO: 34 - protein, 20 aa, Artificial Sequence
  Antigen binding construct or fragment thereof
METDTLLLWVLLLWVPGSTG

SEQ ID NO: 35 - DNA, 54 bp, Artificial Sequence
  Antigen binding construct or fragment thereof
ggctccacatccggcggaggctctggcggtggatctggcggaggcggctcatcc

SEQ ID NO: 36 - protein, 18 aa, Artificial Sequence
  Antigen binding construct or fragment thereof
GSTSGGGSGGGSGGGGSS

SEQ ID NO: 37 - DNA, 393 bp, Artificial Sequence
  Antigen binding construct or fragment thereof
gagcctaagtcctgcgacaagacccacacctgtcccccttgcggcggaggaagcagcggaggcggatccggtggccagcctcgggagcctcaggtgtacaccctgcctccctcccgggacgagctgaccaagaaccaggtgtccctgacctgtctggtcaagggcttctacccttccgatatcgccgtggagtgggagtccaacggccagcctgagaacaactacaagaccacccctcctgtgctggactccgacggctccttcttcctgtactccaagctcacagtggataagtcccggtggcagcagggcaacgtgttctcctgctccgtgatgcacgaggccctgcacaaccactatacccagaagtccctgtccctgtctcctggcaag

SEQ ID NO: 38 - protein, 131 aa, Artificial Sequence
  Antigen binding construct or fragment thereof
EPKSCDKTHTCPPCGGGSSGGGSGGQPREPQVYTLPPSRDELTKNQVSLTCLVKGFYPSDIAVEWESNGQPENNYKTTPPVLDSDGSFFLYSKLTVDKSRWQQGNVFSCSVMHEALHNHYTQKSLSLSPGK

SEQ ID NO: 39 - DNA, 321 bp, Murine
gatgtccagataaaccagtctccatcttttcttgctgcgtctcctggagaaaccattactataaattgcaggacaagtaggagtattagtcaatatttagcctggtatcaagagaaacctgggaaaactaataagcttcttatctactctggatccactctgcaatctggaattccatcaaggttcagtggcagtggatctggtacagatttcactctcaccatcagtggcctggagcctgaagattttgcaatgtattactgtcaacagcataatgaaaacccgctcacgttcggtgctgggaccaagctggagctgaag

SEQ ID NO: 40 - protein, 107 aa, Murine; identical to SEQ ID NO: 7

SEQ ID NO: 41 - DNA, 321 bp, Artificial Sequence
  Antigen binding construct or fragment thereof
gacgtccagataacccagtctccatcctccctgtctgcatctgtaggagacagagtcaccatcacttgcaggacaagtaggagtattagtcaatatttagcctggtatcagcagaaaccagggaaagttcctaagctcctgatctattctggatccactctgcaatctggagtcccatctcggttcagtggcagtggatctgggacagatttcactctcaccatcagcagcctgcagcctgaagatgttgcaacttattactgtcaacagcataatgaaaacccgctcacgttcggcggagggaccaaggtggagatcaaa

SEQ ID NO: 42 - protein, 107 aa, Artificial Sequence; identical to SEQ ID NO: 9
  Antigen binding construct or fragment thereof

SEQ ID NO: 43 - DNA, 354 bp, Murine
gaggtccagctgcagcagtctggggcagagcttgtgaagccaggggcctcagtcaagttgtcctgcacagcttctggcttcaacattaaagacacctatatacacttcgtgaggcagaggcctgaacagggcctggagtggattggaaggattgatcctgcgaatgataatactttatatgcctcaaagttccagggcaaggccactataacagcagacacatcatccaacacagcctacatgcacctctgcagcctgacatctggggacactgccgtctattactgtggtagaggttatggttactacgtatttgaccactggggccaaggcaccactctcacagtctcctca

SEQ ID NO: 44 - protein, 118 aa, Murine; identical to SEQ ID NO: 1

SEQ ID NO: 45 - DNA, 354 bp, Artificial Sequence
  Antigen binding construct or fragment thereof
gaagtgcagctggtggaaagcggcggcggcctggtgcagccgggcggcagcctgcgcctgagctgcgcggcgagcggctttaacattaaagatacctatattcattttgtgcgccaggcgccgggcaaaggcctggaatggattggccgcattgatccggcgaacgataacaccctgtatgcgagcaaatttcagggcaaagcgaccattagcgcggataccagcaaaaacaccgcgtatctgcagatgaacagcctgcgcgcgggagataccgcggtgtattattgcggccgcggctatggctattatgtgtttgatcattggggccagggcaccctggtgaccgtgagcagc

SEQ ID NO: 46 - protein, 118 aa, Artificial Sequence
  Antigen binding construct or fragment thereof
EVQLVESGGGLVQPGGSLRLSCAASGFNIKDTYIHFVRQAPGKGLEWIGRIDPANDNTLYASKFQGKATISADTSKNTAYLQMNSLRAGDTAVYYCGRGYGYYVFDHWGQGTLVTVSS

SEQ ID NO: 47 - DNA, 354 bp, Artificial Sequence
  Antigen binding construct or fragment thereof
gaagtgcagctggtggaaagcggcggcggcctggtgcagccgggcggcagcctgcgcctgagctgcgcggcgagcggctttaacattaaagatacctatattcattttgtgcgccaggcgccgggcaaaggcctggaatggattggccgcattgatccggcgaacgataacaccctgtatgcgagcaaatttcagggcaaagcgaccattagcgcggataccagcaaaaacaccgcgtatctgcagatgaacagcctgcgcgcggaagataccgcggtgtattattgcggccgcggctatggctattatgtgtttgatcattggggccagggcaccctggtgaccgtgagcagc

SEQ ID NO: 48 - protein, 118 aa, Artificial Sequence
  Antigen binding construct or fragment thereof
EVQLVESGGGLVQPGGSLRLSCAASGFNIKDTYIHFVRQAPGKGLEWIGRIDPANDNTLYASKFQGKATISADTSKNTAYLQMNSLRAEDTAVYYCGRGYGYYVFDHWGQGTLVTVSS

SEQ ID NO: 49 - DNA, 354 bp, Artificial Sequence
  Antigen binding construct or fragment thereof
caggtgcagctggtgcagagcggcgcggaagtgaaaaaaccgggcgcgaccgtgaaaattagctgcaaagtgagcggctttaacattaaagatacctatattcattttgtgcagcaggcgccgggcaaaggcctggaatggattggccgcattgatccggcgaacgataacaccctgtatgcgagcaaatttcagggcaaagcgaccattaccgcggataccagcaccgataccgcgtatatggaactgagcagcctgcgcagcggagataccgcggtgtattattgcggccgcggctatggctattatgtgtttgatcattggggccagggcaccctggtgaccgtgagcagc

SEQ ID NO: 50 - protein, 118 aa, Artificial Sequence
  Antigen binding construct or fragment thereof
QVQLVQSGAEVKKPGATVKISCKVSGFNIKDTYIHFVQQAPGKGLEWIGRIDPANDNTLYASKFQGKATITADTSTDTAYMELSSLRSGDTAVYYCGRGYGYYVFDHWGQGTLVTVSS

SEQ ID NO: 51 - DNA, 354 bp, Artificial Sequence
  Antigen binding construct or fragment thereof
caggtgcagctggtgcagagcggcgcggaagtgaaaaaaccgggcgcgaccgtgaaaattagctgcaaagtgagcggctttaacattaaagatacctatattcattttgtgcagcaggcgccgggcaaaggcctggaatggattggccgcattgatccggcgaacgataacaccctgtatgcgagcaaatttcagggcaaagcgaccattaccgcggataccagcaccgataccgcgtatatggaactgagcagcctgcgcagcgaagataccgcggtgtattattgcggccgcggctatggctattatgtgtttgatcattggggccagggcaccctggtgaccgtgagcagc

SEQ ID NO: 52 - protein, 117 aa, Artificial Sequence
  Antigen binding construct or fragment thereof
QVQLVQSGAEVKKPGATVKISCKVSGFNIKDTYIHFVQQAPGKGLEWIGRIDPANDNTLYASKFQGKATITADTSTDTAYMELSSLRSEDTAVYYCGRGYGYYVFDHWGQGTLVTVS

SEQ ID NO: 53 - protein, 23 aa, Artificial Sequence
  Antigen binding construct or fragment thereof
EPKSCDKTHTCPPCPAPELLGGP

SEQ ID NO: 54 - protein, 25 aa, Artificial Sequence
  Antigen binding construct or fragment thereof
EPKSCDKTHTCPPCPGGGSSGGGSG

SEQ ID NO: 55 - protein, 19 aa, Artificial Sequence
  Antigen binding construct or fragment thereof
ERKCCVECPPCPAPPVAGP

SEQ ID NO: 56 - protein, 70 aa, Artificial Sequence
  Antigen binding construct or fragment thereof
ELKTPLGDTTHTCPRCPEPKSCDTPPPCPRCPEPKSCDTPPPCPRCPEPKSCDTPPPCPRCPAPELLGGP

SEQ ID NO: 57 - protein, 25 aa, Artificial Sequence
  Antigen binding construct or fragment thereof
ELKTPLGDTTHTCPRCPAPELLGGP

SEQ ID NO: 58 - protein, 23 aa, Artificial Sequence
  Antigen binding construct or fragment thereof
EPKSCDTPPPCPRCPAPELLGGP

SEQ ID NO: 59 - protein, 20 aa, Artificial Sequence
  Antigen binding construct or fragment thereof
ESKYGPPCPSCPAPEFLGGP

SEQ ID NO: 60 - protein, 20 aa, Artificial Sequence
  Antigen binding construct or fragment thereof
ESKYGPPCPPCPAPEFLGGP

SEQ ID NO: 61 - DNA, 15 bp, Artificial Sequence
  Restriction site
tctagagccgccacc

SEQ ID NO: 62 - DNA, 15 bp, Artificial Sequence
  Restriction site
tctagagccgccacc

SEQ ID NO: 63 - DNA, 6 bp, Artificial Sequence
  Restriction site
aagctt

SEQ ID NO: 64 - DNA, 6 bp, Artificial Sequence
  Restriction site
aagctt

SEQ ID NO: 65 - DNA, 15 bp, Artificial Sequence
  Restriction site
tctagagccgccacc

SEQ ID NO: 66 - DNA, 6 bp, Artificial Sequence
  Restriction site
aagctt

SEQ ID NO: 67 - DNA, 15 bp, Artificial Sequence
  Restriction site
tctagagccgccacc

SEQ ID NO: 68 - DNA, 6 bp, Artificial Sequence
  Restriction site
aagctt

SEQ ID NO: 69 - DNA, 15 bp, Artificial Sequence
  Restriction site
tctagagccgccacc

SEQ ID NO: 70 - DNA, 6 bp, Artificial Sequence
  Restriction site
aagctt

SEQ ID NO: 71 - DNA, 15 bp, Artificial Sequence
  Restriction site
tctagagccgccacc

SEQ ID NO: 72 - DNA, 6 bp, Artificial Sequence
  Restriction site
aagctt

SEQ ID NO: 73 - DNA, 15 bp, Artificial Sequence
  Restriction site
tctagagccgccacc

SEQ ID NO: 74 - DNA, 6 bp, Artificial Sequence
  Restriction site
aagctt

SEQ ID NO: 75 - DNA, 15 bp, Artificial Sequence
  Restriction site
tctagagccgccacc

SEQ ID NO: 76 - DNA, 6 bp, Artificial Sequence
  Restriction site
aagctt

SEQ ID NO: 77 - DNA, 759 bp, Artificial Sequence
  Antigen binding construct or fragment thereof
atggagaccgatacactgctgctgtgggtgctgctgctctgggtccctggcagcacaggagacatccagatgacacagagccctagctccctgagcgcttccgtgggagatagggtgaccatcacatgccggacctccaggtccatctcccagtacctggcctggtaccagcagaagcccggcaaggtgcccaagctgctcatctatagcggcagcaccctgcagagcggagtgccttcccggttttccggatccggctccggcacagactttaccctgaccatctccagcctgcagcctgaggatgtcgccacctactactgccaacagcacaacgagaaccccctgaccttcggcggcggaaccaaggtcgagatcaagtccggaggaggaggccaagtgcagctggtccaatccggcgccgaagtgaaaaagcccggcgccaccgtgaagatcagctgcaaggtgtccggcttcaacatcaaggacacctatatccactgggtccagcaagcccccggaaaaggcctggagtggatgggacggattgaccccgccaacgacaacacactctatgcctccaagttccagggcagggtgacaatcaccgccgacaccagcaccgacacagcttatatggagctgtcctccctccggtccgaggataccgccgtctactactgcgccaggggctacggctactacgtgtttgaccactggggccagggcaccctggtgacagtgtccagcggaggctgc

SEQ ID NO: 78 - DNA, 759 bp, Artificial Sequence
  Antigen binding construct or fragment thereof
atggagaccgacaccctgctgctctgggtcctcctgctgtgggtgcctggcagcacaggacaggtgcaactggtgcagagcggcgccgaggtcaagaaacctggcgccaccgtgaagatcagctgcaaggtgtccggcttcaacatcaaggacacctacatccactgggtccaacaagcccccggaaagggcctggaatggatgggccggattgaccccgccaacgacaacaccctctatgccagcaagttccagggcagggtcaccatcaccgccgacaccagcaccgacaccgcctacatggagctgagcagcctgcggagcgaagacaccgccgtgtactactgcgccaggggctacggctactacgtcttcgaccattggggacagggcaccctcgtgacagtgtccagctccggcggaggaggagatatccagatgacccagagcccttccagcctgtccgcttccgtgggagatcgggtgaccatcacatgcaggacctccaggtccatctcccagtacctggcctggtaccaacagaagcccggcaaggtgcccaagctgctgatctacagcggcagcacactgcaatccggcgtcccttcccggttttccggatccggatccggcaccgacttcaccctgaccatcagctccctgcaacccgaggacgtggccacctactactgtcagcagcacaacgagaaccccctcacctttggcggcggaaccaaggtcgagatcaagggcggctgc

SEQ ID NO: 79 - protein, 22 aa, Artificial Sequence
  Antigen binding construct or fragment thereof
ERKCCVECPPCPGGGSSGGGSG

SEQ ID NO: 80 - protein, 107 aa, Artificial Sequence
  Antigen binding construct or fragment thereof
GQPREPQVYTLPPSREEMTKNQVSLTCLVKGFYPSDIAVEWESNGQPENNYKTTPPMLDSDGSFFLYSKLTVDKSRWQQGNVFSCSVMHEALHNHYTQKSLSLSPGK

SEQ ID NO: 81 - protein, 107 aa, Artificial Sequence
  Antigen binding construct or fragment thereof
GQPREPQVYTLPPSRDELTKNQVSLTCLVKGFYPSDIAVEWESNGQPENNYKTTPPVLDSDGSFFLYSKLTVDKSRWQQGNVFSCSVMHEALHNHYTQKSLSLSPGK